European Patent Specification EP 3 687 287 B1, published July 12, 2023. Title: Non-Human Animals Expressing Humanized C1Q Complex. Applicant: Regeneron Pharmaceuticals, Inc. The sequence listing filed with the application follows.

SEQUENCE LISTING (94 sequences)

SEQ ID NO: 1 - protein, 245 aa, Mus musculus
METSQGWLVACVLTMTLVWTVAEDVCRAPNGKDGAPGNPGRPGRPGLKGERGEPGAAGIRTGIRGFKGDPGESGPPGKPGNVGLPGPSGPLGDSGPQGLKGVKGNPGNIRDQPRPAFSAIRQNPMTLGNVVIFDKVLTNQESPYQNHTGRFICAVPGFYYFNFQVISKWDLCLFIKSSSGGQPRDSLSFSNTNNKGLFQVLAGGTVLQLRRGDEVWIEKDPAKGRIYQGTEADSIFSGFLIFPSA

SEQ ID NO: 2 - protein, 253 aa, Mus musculus
MKTQWGEVWTHLLLLLLGFLHVSWAQSSCTGPPGIPGIPGVPGVPGSDGQPGTPGIKGEKGLPGLAGDLGEFGEKGDPGIPGTPGKVGPKGPVGPKGTPGPSGPRGPKGDSGDYGATQKVAFSALRTINSPLRPNQVIRFEKVITNANENYEPRNGKFTCKVPGLYYFTYHASSRGNLCVNLVRGRDRDSMQKVVTFCDYAQNTFQVTTGGVVLKLEQEEVVHLQATDKNSLLGIEGANSIFTGFLLFPDMDA

SEQ ID NO: 3 - protein, 246 aa, Mus musculus
MVVGPSCQPPCGLCLLLLFLLALPLRSQASAGCYGIPGMPGMPGAPGKDGHDGLQGPKGEPGIPAVPGTRGPKGQKGEPGMPGHRGKNGPRGTSGLPGDPGPRGPPGEPGVEGRYKQKHQSVFTVTRQTTQYPEANALVRFNSVVTNPQGHYNPSTGKFTCEVPGLYYFVYYTSHTANLCVHLNLNLARVASFCDHMFNSKQVSSGGVLLRLQRGDEVWLSVNDYNGMVGIEGSNSVFSGFLLFPD

SEQ ID NO: 4 - protein, 245 aa, Homo sapiens
MEGPRGWLVLCVLAISLASMVTEDLCRAPDGKKGEAGRPGRRGRPGLKGEQGEPGAPGIRTGIQGLKGDQGEPGPSGNPGKVGYPGPSGPLGARGIPGIKGTKGSPGNIKDQPRPAFSAIRRNPPMGGNVVIFDTVITNQEEPYQNHSGRFVCTVPGYYYFTFQVLSQWEICLSIVSSSRGQVRRSLGFCDTTNKGLFQVVSGGMVLQLQQGDQVWVEKDPKKGHIYQGSEADSVFSGFLIFPSA

SEQ ID NO: 5 - protein, 251 aa, Homo sapiens
MKIPWGSIPVLMLLLLLGLIDISQAQLSCTGPPAIPGIPGIPGTPGPDGQPGTPGIKGEKGLPGLAGDHGEFGEKGDPGIPGNPGKVGPKGPMGPKGGPGAPGAPGPKGESGDYKATQKIAFSATRTINVPLRRDQTIRFDHVITNMNNNYEPRSGKFTCKVPGLYYFTYHASSRGNLCVNLMRGRERAQKVVTFCDYAYNTFQVTTGGMVLKLEQGENVFLQATDKNSLLGMEGANSIFSGFLLFPDMEA

SEQ ID NO: 6 - protein, 245 aa, Homo sapiens
MDVGPSSLPHLGLKLLLLLLLLPLRGQANTGCYGIPGMPGLPGAPGKDGYDGLPGPKGEPGIPAIPGIRGPKGQKGEPGLPGHPGKNGPMGPPGMPGVPGPMGIPGEPGEEGRYKQKFQSVFTVTRQTHQPPAPNSLIRFNAVLTNPQGDYDTSTGKFTCKVPGLYYFVYHASHTANLCVLLYRSGVKVVTFCGHTSKTNQVNSGGVLLRLQVGEEVWLAVNDYYDMVGIQGSDSVFSGFLLFPD

SEQ ID NO: 7 - protein, 245 aa, Rattus norvegicus
METSQGWLVACVLAVTLVWTVAEDVCRAPNGKDGVAGIPGRPGRPGLKGERGEPGAAGIRTGIRGLKGDMGESGPPGKPGNVGFPGPTGPLGNSGPQGLKGVKGNPGNIRDQPRPAFSAIRQNPPTYGNVVVFDKVLTNQENPYQNRTGHFICAVPGFYYFTFQVISKWDLCLSIVSSSRGQPRNSLGFCDTNSKGLFQVLAGGTVLQLQRGDEVWIEKDPAKGRIYQGTEADSIFSGFLIFPSA

SEQ ID NO: 8 - protein, 253 aa, Rattus norvegicus
MKTQWSEILTPLLLLLLGLLHVSWAQSSCTGSPGIPGVPGIPGVPGSDGKPGTPGIKGEKGLPGLAGDHGELGEKGDAGIPGIPGKVGPKGPVGPKGAPGPPGPRGPKGDSGDYKATQKVAFSALRTVNSALRPNQAIRFEKVITNVNDNYEPRSGKFTCKVPGLYYFTYHASSRGNLCVNIVRGRDRDRMQKVLTFCDYAQNTFQVTTGGVVLKLEQEEVVHLQATDKNSLLGVEGANSIFTGFLLFPDMDV

SEQ ID NO: 9 - protein, 248 aa, Rattus norvegicus
MLRMVVGTSCQPQHGLYLLLLLLALPLRSQANAGCYGIPGMPGLPGTPGKDGHDGLQGPKGEPGIPAIPGTQGPKGQKGEPGMPGHRGKNGPMGTSGSPGDPGPRGPPGEPGEEGRYKQKHQSVFTVTRQTAQYPAANGLVKFNSAITNPQGDYNTNTGKFTCKVPGLYYFVHHTSQTANLCVQLLLNNAKVTSFCDHMSNSKQVSSGGVLLRLQRGDEVWLAVNDYNGMVGTEGSDSVFSGFLLFPD

SEQ ID NO: 10 - protein, 245 aa, Artificial Sequence
  polypeptide sequence of a chimeric mouse/human C1qa
METSQGWLVACVLTMTLVWTVAEDVCRAPNGKDGAPGNPGRPGRPGLKGERGEPGAAGIRTGIRGFKGDPGESGPPGKPGNVGLPGPTGPLGDSGPQGLKGVKGNPGNIRDQPRPAFSAIRRNPPMGGNVVIFDTVITNQEEPYQNHSGRFVCTVPGYYYFTFQVLSQWEICLSIVSSSRGQVRRSLGFCDTTNKGLFQVVSGGMVLQLQQGDQVWVEKDPKKGHIYQGSEADSVFSGFLIFPSA

SEQ ID NO: 11 - protein, 251 aa, Artificial Sequence
  polypeptide sequence of a chimeric mouse/human C1qb
MKTQWGEVWTHLLLLLLGFLHVSWAQSSCTGPPGIPGIPGVPGVPGSDGQPGTPGIKGEKGLPGLAGDLGEFGEKGDPGIPGTPGKVGPKGPVGPKGTPGPSGPRGPKGDSGDYGATQKIAFSATRTINVPLRRDQTIRFDHVITNMNNNYEPRSGKFTCKVPGLYYFTYHASSRGNLCVNLMRGRERAQKVVTFCDYAYNTFQVTTGGMVLKLEQGENVFLQATDKNSLLGMEGANSIFSGFLLFPDMEA

SEQ ID NO: 12 - protein, 246 aa, Artificial Sequence
  polypeptide sequence of a chimeric mouse/human C1qc
MVVGPSCQPPCGLCLLLLFLLALPLRSQASAGCYGIPGMPGMPGAPGKDGHDGLQGPKGEPGIPAVPGTRGPKGQKGEPGMPGHRGKNGPRGTSGLPGDPGPRGPPGEPGVEGRYKQKFQSVFTVTRQTHQPPAPNSLIRFNAVLTNPQGDYDTSTGKFTCKVPGLYYFVYHASHTANLCVLLYRSGVKVVTFCGHTSKTNQVNSGGVLLRLQVGEEVWLAVNDYYDMVGIQGSDSVFSGFLLFPD

SEQ ID NO: 13 - DNA, 67 bp, Artificial Sequence
  synthetic oligonucleotide
catacccagtgtccctgtgtgtctctgtagggacaccatgggtaccgatttaaatgatccagtggtc

SEQ ID NO: 14 - DNA, 73 bp, Artificial Sequence
  synthetic oligonucleotide
gcagcccctagataacttcgtataatgtatgctatacgaagttatcctaggctatccaacaccatcttcctgc

SEQ ID NO: 15 - DNA, 23 bp, Artificial Sequence
  synthetic oligonucleotide
tcccgcaccatcctggaggcaat

SEQ ID NO: 16 - DNA, 20 bp, Artificial Sequence
  synthetic oligonucleotide
taagcgttctctccggctgg

SEQ ID NO: 17 - DNA, 21 bp, Artificial Sequence
  synthetic oligonucleotide
cgcttctcaggacccctaaac

SEQ ID NO: 18 - DNA, 27 bp, Artificial Sequence
  synthetic oligonucleotide
cgatactgtcgtcgtcccctcaaactg

SEQ ID NO: 19 - DNA, 20 bp, Artificial Sequence
  synthetic oligonucleotide
ggagtgcgatcttcctgagg

SEQ ID NO: 20 - DNA, 19 bp, Artificial Sequence
  synthetic oligonucleotide
cgcatcgtaaccgtgcatc

SEQ ID NO: 21 - DNA, 23 bp, Artificial Sequence
  synthetic oligonucleotide
tgggcacaacagacaatcggctg

SEQ ID NO: 22 - DNA, 19 bp, Artificial Sequence
  synthetic oligonucleotide
ggtggagaggctattcggc

SEQ ID NO: 23 - DNA, 17 bp, Artificial Sequence
  synthetic oligonucleotide
gaacacggcggcatcag

SEQ ID NO: 24 - DNA, 25 bp, Artificial Sequence
  synthetic oligonucleotide
aggaccatcaacagccccttgcgac

SEQ ID NO: 25 - DNA, 20 bp, Artificial Sequence
  synthetic oligonucleotide
gaaagtcgccttctctgccc

SEQ ID NO: 26 - DNA, 20 bp, Artificial Sequence
  synthetic oligonucleotide
cgaagcgaatgacctggttc

SEQ ID NO: 27 - DNA, 27 bp, Artificial Sequence
  synthetic oligonucleotide
tgacaaggtcctcaccaaccaggagag

SEQ ID NO: 28 - DNA, 19 bp, Artificial Sequence
  probe
cgcttggcaacgtggttat

SEQ ID NO: 29 - DNA, 20 bp, Artificial Sequence
  synthetic oligonucleotide
cccgtgtggttctggtatgg

SEQ ID NO: 30 - DNA, 25 bp, Artificial Sequence
  synthetic oligonucleotide
tatgagccacgcaacggcaagttca

SEQ ID NO: 31 - DNA, 19 bp, Artificial Sequence
  synthetic oligonucleotide
tcaccaacgcgaacgagaa

SEQ ID NO: 32 - DNA, 16 bp, Artificial Sequence
  synthetic oligonucleotide
ggccaggcaccttgca

SEQ ID NO: 33 - DNA, 28 bp, Artificial Sequence
  synthetic oligonucleotide
cccatcctcactcagacctcttcctcca

SEQ ID NO: 34 - DNA, 19 bp, Artificial Sequence
  synthetic oligonucleotide
cacctcgctccctctgctt

SEQ ID NO: 35 - DNA, 20 bp, Artificial Sequence
  synthetic oligonucleotide
caggaaccagggtggacttc

SEQ ID NO: 36 - DNA, 26 bp, Artificial Sequence
  synthetic oligonucleotide
caacgtggtcatcttcgacacggtca

SEQ ID NO: 37 - DNA, 16 bp, Artificial Sequence
  synthetic oligonucleotide
cggaaccccccaatgg

SEQ ID NO: 38 - DNA, 22 bp, Artificial Sequence
  synthetic oligonucleotide
tggttctggtacggttcttcct

SEQ ID NO: 39 - DNA, 21 bp, Artificial Sequence
  synthetic oligonucleotide
accatcaacgtccccctgcgc

SEQ ID NO: 40 - DNA, 20 bp, Artificial Sequence
  synthetic oligonucleotide
aatcgccttctctgccacaa

SEQ ID NO: 41 - DNA, 18 bp, Artificial Sequence
  probe
gtggtcgaagcggatggt

SEQ ID NO: 42 - DNA, 22 bp, Artificial Sequence
  synthetic oligonucleotide
cacctgcaaagtccccggcctc

SEQ ID NO: 43 - DNA, 20 bp, Artificial Sequence
  synthetic oligonucleotide
tgacacgagcactggcaagt

SEQ ID NO: 44 - DNA, 22 bp, Artificial Sequence
  synthetic oligonucleotide
cgacgcgtggtagacaaagtag

SEQ ID NO: 45 - DNA, 21 bp, Artificial Sequence
  synthetic oligonucleotide
acgagcgggttcggcccattc

SEQ ID NO: 46 - DNA, 17 bp, Artificial Sequence
  synthetic oligonucleotide
tgcggccgatcttagcc

SEQ ID NO: 47 - DNA, 18 bp, Artificial Sequence
  synthetic oligonucleotide
ttgaccgattccttgcgg

SEQ ID NO: 48 - DNA, 103 bp, Artificial Sequence
  synthetic oligonucleotide
cggcccccaaggactgaagggcgtgaaaggcaatccaggcaatatcagggaccagccgaggccagccttctccgccattcggcggaaccccccaatggggggc

SEQ ID NO: 49 - DNA, 104 bp, Artificial Sequence
  synthetic oligonucleotide
ttgagagggaggcctaagaataataacaatccagtgcttaagagtcaggcgcgatcgctgatgcacgcctttaatcccagcacttgggaggcagagacaggtga

SEQ ID NO: 50 - DNA, 105 bp, Artificial Sequence
  synthetic oligonucleotide
gccaggggacccaggccccagggggcctccgggggagccaggtgtggagggccgatacaagcagaaattccagtcagtgttcacggtcactcggcagacccacca

SEQ ID NO: 51 - DNA, 99 bp, Artificial Sequence
  synthetic oligonucleotide
tgaatttcggatcttcaactttgcatcagccatagctgggctctggactctacctaactataacggtcctaaggtagcgaaagggggatgatttggagt

SEQ ID NO: 52 - DNA, 110 bp, Artificial Sequence
  synthetic oligonucleotide
tccaggcccctctggaccccgcggtcccaaaggcgattctggggactacggggctacacagaaaatcgccttctctgccacaagaaccatcaacgtccccctgcgccggg

SEQ ID NO: 53 - DNA, 101 bp, Artificial Sequence
  synthetic oligonucleotide
gcacctggcacaccagaagtgccatgctcagaaatgttggttacatgaatgaatgcggccgcaccggtataacttcgtataatgtatgctatacgaagtta

SEQ ID NO: 54 - DNA, 101 bp, Artificial Sequence
  synthetic oligonucleotide
ccggcgcgccataacttcgtataatgtatgctatacgaagttatgtcgacgaatgttcataggctggggagatggctcagtcagtaaagtacttagcttgc

SEQ ID NO: 55 - protein, 245 aa, Artificial Sequence
  polypeptide sequence of a chimeric rat/human C1qa
METSQGWLVACVLAVTLVWTVAEDVCRAPNGKDGVAGIPGRPGRPGLKGERGEPGAAGIRTGIRGLKGDMGESGPPGKPGNVGFPGPTGPLGNSGPQGLKGVKGNPGNIRDQPRPAFSAIRRNPPMGGNVVIFDTVITNQEEPYQNHSGRFVCTVPGYYYFTFQVLSQWEICLSIVSSSRGQVRRSLGFCDTTNKGLFQVVSGGMVLQLQQGDQVWVEKDPKKGHIYQGSEADSVFSGFLIFPSA

SEQ ID NO: 56 - protein, 251 aa, Artificial Sequence
  polypeptide sequence of a chimeric rat/human C1qb
MKTQWSEILTPLLLLLLGLLHVSWAQSSCTGSPGIPGVPGIPGVPGSDGKPGTPGIKGEKGLPGLAGDHGELGEKGDAGIPGIPGKVGPKGPVGPKGAPGPPGPRGPKGDSGDYKATQKIAFSATRTINVPLRRDQTIRFDHVITNMNNNYEPRSGKFTCKVPGLYYFTYHASSRGNLCVNLMRGRERAQKVVTFCDYAYNTFQVTTGGMVLKLEQGENVFLQATDKNSLLGMEGANSIFSGFLLFPDMEA

SEQ ID NO: 57 - protein, 248 aa, Artificial Sequence
  polypeptide sequence of a chimeric rat/human C1qc
MLRMVVGTSCQPQHGLYLLLLLLALPLRSQANAGCYGIPGMPGLPGTPGKDGHDGLQGPKGEPGIPAIPGTQGPKGQKGEPGMPGHRGKNGPMGTSGSPGDPGPRGPPGEPGEEGRYKQKFQSVFTVTRQTHQPPAPNSLIRFNAVLTNPQGDYDTSTGKFTCKVPGLYYFVYHASHTANLCVLLYRSGVKVVTFCGHTSKTNQVNSGGVLLRLQVGEEVWLAVNDYYDMVGIQGSDSVFSGFLLFPD

SEQ ID NO: 58 - DNA, 103 bp, Artificial Sequence
  synthetic oligonucleotide
gattctcccaatctctcctctgcaggaccactggatcatttaaatcggtacccatgatgttcctgcagagacacacagggaccccgggcatgctggacagtca

SEQ ID NO: 59 - DNA, 101 bp, Artificial Sequence
  synthetic oligonucleotide
tagttatcgagcccggggatccactagttctagtgtttaaactctagccgggggatccagacatgataagatacattgatgagtttggacaaaccacaact

SEQ ID NO: 60 - DNA, 101 bp, Artificial Sequence
  synthetic oligonucleotide
aggattactggcagggaggaggttttggataggagtgatttgaccccgtgagctagcataacttcgtatagcatacattatacgaagttatctaggggctg

SEQ ID NO: 61 - DNA, 23 bp, Artificial Sequence
  synthetic oligonucleotide
aacccaccgacgtatggcaacgt

SEQ ID NO: 62 - DNA, 21 bp, Artificial Sequence
  synthetic oligonucleotide
gccagctttctcagctattcg

SEQ ID NO: 63 - DNA, 21 bp, Artificial Sequence
  synthetic oligonucleotide
gcggttctggtatggattctc

SEQ ID NO: 64 - DNA, 24 bp, Artificial Sequence
  synthetic oligonucleotide
aaacaccttccaggtcaccacggg

SEQ ID NO: 65 - DNA, 21 bp, Artificial Sequence
  synthetic oligonucleotide
tctcaccttctgcgactatgc

SEQ ID NO: 66 - DNA, 22 bp, Artificial Sequence
  synthetic oligonucleotide
cctgctccagcttcaagactac

SEQ ID NO: 67 - DNA, 21 bp, Artificial Sequence
  synthetic oligonucleotide
acgagcgggttcggcccattc

SEQ ID NO: 68 - DNA, 17 bp, Artificial Sequence
  synthetic oligonucleotide
tgcggccgatcttagcc

SEQ ID NO: 69 - DNA, 18 bp, Artificial Sequence
  synthetic oligonucleotide
ttgaccgattccttgcgg

SEQ ID NO: 70 - DNA, 27 bp, Artificial Sequence
  synthetic oligonucleotide
cgatactgtcgtcgtcccctcaaactg

SEQ ID NO: 71 - DNA, 20 bp, Artificial Sequence
  synthetic oligonucleotide
ggagtgcgatcttcctgagg

SEQ ID NO: 72 - DNA, 19 bp, Artificial Sequence
  synthetic oligonucleotide
cgcatcgtaaccgtgcatc

SEQ ID NO: 73 - DNA, 23 bp, Artificial Sequence
  synthetic oligonucleotide
aacccaccgacgtatggcaacgt

SEQ ID NO: 74 - DNA, 21 bp, Artificial Sequence
  synthetic oligonucleotide
gccagctttctcagctattcg

SEQ ID NO: 75 - DNA, 21 bp, Artificial Sequence
  synthetic oligonucleotide
gcggttctggtatggattctc

SEQ ID NO: 76 - DNA, 24 bp, Artificial Sequence
  synthetic oligonucleotide
aaacaccttccaggtcaccacggg

SEQ ID NO: 77 - DNA, 21 bp, Artificial Sequence
  synthetic oligonucleotide
tctcaccttctgcgactatgc

SEQ ID NO: 78 - DNA, 22 bp, Artificial Sequence
  synthetic oligonucleotide
cctgctccagcttcaagactac

SEQ ID NO: 79 - DNA, 22 bp, Artificial Sequence
  synthetic oligonucleotide
ccttccaggtgctgtcccagtg

SEQ ID NO: 80 - DNA, 22 bp, Artificial Sequence
  synthetic oligonucleotide
gtacccggctactactacttca

SEQ ID NO: 81 - DNA, 23 bp, Artificial Sequence
  synthetic oligonucleotide
gagacgatggacaggcagatttc

SEQ ID NO: 82 - DNA, 21 bp, Artificial Sequence
  synthetic oligonucleotide
accatcaacgtccccctgcgc

SEQ ID NO: 83 - DNA, 20 bp, Artificial Sequence
  synthetic oligonucleotide
aatcgccttctctgccacaa

SEQ ID NO: 84 - DNA, 18 bp, Artificial Sequence
  synthetic oligonucleotide
gtggtcgaagcggatggt

SEQ ID NO: 85 - DNA, 22 bp, Artificial Sequence
  synthetic oligonucleotide
cacctgcaaagtccccggcctc

SEQ ID NO: 86 - DNA, 20 bp, Artificial Sequence
  synthetic oligonucleotide
tgacacgagcactggcaagt

SEQ ID NO: 87 - DNA, 22 bp, Artificial Sequence
  synthetic oligonucleotide
cgacgcgtggtagacaaagtag

SEQ ID NO: 88 - DNA, 102 bp, Artificial Sequence
  synthetic oligonucleotide
gcccccaagggttgaaaggtgtgaaaggcaatccgggcaatatcagggaccagccgaggccagccttctccgccattcggcggaaccccccaatggggggca

SEQ ID NO: 89 - DNA, 106 bp, Artificial Sequence
  synthetic oligonucleotide
gcattgagagggaggcctaagaataataacaatccagtgcttaagagtcaggcgctgggtagctgccccacgttctgccatctcctgcactccctgttgcggggcc

SEQ ID NO: 90 - DNA, 105 bp, Artificial Sequence
  synthetic oligonucleotide
gggatccaggccccaggggtcctcccggggagccgggtgaggagggtcgatacaagcagaaattccagtcagtgttcacggtcactcggcagacccaccagcccc

SEQ ID NO: 91 - DNA, 100 bp, Artificial Sequence
  synthetic oligonucleotide
tgaatttcggatcttcaactttgcatcagccatagctgggctctggactcgaatggcaggctgggtccagcacccggacgcccgcctcgctccctctgct

SEQ ID NO: 92 - DNA, 104 bp, Artificial Sequence
  synthetic oligonucleotide
gcccccctggaccccgcggtcccaaaggtgactctggagactacaaggctacccagaaaatcgccttctctgccacaagaaccatcaacgtccccctgcgccgg

SEQ ID NO: 93 - DNA, 101 bp, Artificial Sequence
  synthetic oligonucleotide
ctggcacaccagaagtgccatgctcagaaatgttggttacatgaatgaatgtcgagataacttcgtataatgtatgctatacgaagttatatgcatgccag

SEQ ID NO: 94 - DNA, 132 bp, Artificial Sequence
  synthetic oligonucleotide
ggcggcctagataacttcgtataatgtatgctatacgaagttatgctaggtaactataacggtcctaaggtagcgagctagctcacggggtcaaatcactcctatccaaaacctcctccctgccagtaatcc